European Patent Specification EP 4 402 157 B1, published December 17, 2025. Title: CLEAVABLE LINKERS. Applicant: XILIO THERAPEUTICS. The sequence listing filed with the application follows.

SEQUENCE LISTING (16 sequences)

SEQ ID NO: 1 - protein, 8 aa, synthetic construct
PVSLRSGS

SEQ ID NO: 2 - protein, 10 aa, synthetic construct
GMPKDLYHAS

SEQ ID NO: 3 - protein, 8 aa, synthetic construct
RPLALWRS

SEQ ID NO: 4 - protein, 8 aa, synthetic construct
TQKPLGLS

SEQ ID NO: 5 - protein, 10 aa, synthetic construct
APAGLIVPYN

SEQ ID NO: 6 - protein, 9 aa, synthetic construct
PANLVAPDP

SEQ ID NO: 7 - protein, 10 aa, synthetic construct
IVGRPRHQGV

SEQ ID NO: 8 - protein, 8 aa, synthetic construct
RSKYLATA

SEQ ID NO: 9 - protein, 14 aa, synthetic construct
RVGPVSLRSGSGKI

SEQ ID NO: 10 - protein, 16 aa, synthetic construct
RQGGMPKDLYHASAKQ

SEQ ID NO: 11 - skipped

SEQ ID NO: 12 - protein, 4 aa, synthetic construct
PLGL

SEQ ID NO: 13 - protein, 4 aa, synthetic construct
PLAL

SEQ ID NO: 14 - protein, 4 aa, synthetic construct
PAGL

SEQ ID NO: 15 - protein, 4 aa, synthetic construct
PVSL

SEQ ID NO: 16 - protein, 4 aa, synthetic construct
PANL